European Patent Application EP 4 389 881 A1, published June 26, 2024. Title: Genetisch modifizierter Mikroorganismus und dessen Verwendung zur Herstellung von D-Chiro-Inositol. Applicant: Forschungszentrum Juelich GmbH. The sequence listing filed with the application follows.

SEQUENCE LISTING (51 sequences)

SEQ ID NO: 1 - protein, 319 aa, Medicago truncatula
MSKTVCVTGASGAIGSWVVRLLLERGYTVHATIQDLEDENETKHLEAMEGAKTRLKFFEMDLLNSDSIAAAVKGCAGVIHLACPNIIGEVKDPEKQILEPAIQGTVNVLKVAKEAGVERVVATSSISAIIPSPSWPADKIKAEDCWTDLEYCKEKKLYYPIAKTLAEKAGWEFAKETGFDVVMINPGTALGPLIPPRINSSMAVLAGVLKGDKETYEDFFMGMAHFKDIALAHILGFEQKKASGRHLCVEAIRHYSDFVNLVAELYPEYNVAKIPTDTQPGLLRAKNASKKLIELGLEFTPAEEIIKDAVECLKSRGLV

SEQ ID NO: 2 - protein, 322 aa, Medicago truncatula
MAGNKIPEVLLNSGHKMPVIGMGTSVDNRPSNDVLASIFVDAIKVGYRHFDSASVYGTEEAIGMAVAKALEQGLIKSRDELFITSKPWNTDADYDLIVPALKTTLKKLGTEYVDLYLIHWPVRLRHDLENPVIFTKEDLLPFDIEGTWKAMEECYKLGLAKSIGICNYGTKKLTKLLETATITPAVNQVEMNPSWQQGKLREFCKEKGIHVSAWSALGAYKVTWGSGAVVENQILQDIAAAKGKTTAQVALRWVYQIGSSAMAKSFNKERMTQNLEIFDFELSEDDLEKIKQIPQRRQYLGDMWLSENGSCKTLEELWDGDV

SEQ ID NO: 3 - DNA, 960 bp, Medicago truncatula
  source 1..960: mol_type = genomic DNA
atgtcaaagacagtttgtgtgaccggagccagcggagccatcggatcatgggtggttcgcctcctcctcgaacgaggctacaccgtccatgccaccatccaagatcttgaggatgaaaatgagacaaagcatttggaagcaatggaaggagcaaagactcgtctcaaattttttgaaatggatcttcttaacagtgactctatcgcggccgccgtgaaaggctgtgccggtgttatacacctggcatgtcctaacatcatcggtgaagtcaaggaccccgagaagcaaattttggaaccggcaattcaaggaacggttaacgtgttgaaggttgcaaaggaagcaggggtggagcgtgtggtggcgacgtcgtcgatctccgccatcataccgagtcctagctggccagctgataagattaaggcagaggattgttggacggaccttgaatattgcaaggaaaagaagttatactaccccattgcaaagacactagcagaaaaagctggttgggaatttgctaaagagactggttttgatgtggtcatgattaaccctggtacagcattgggccctttgattccaccaagaattaactcaagcatggctgtacttgctggtgttctcaaaggtgacaaagagacatatgaggacttcttcatgggaatggctcattttaaagacatagctttggcacatattttgggatttgagcaaaagaaagcatctggaaggcatttgtgtgtggaagctattcgtcactatagtgattttgtgaatttggttgcagagttataccctgaatataatgtggcaaagataccaacggatactcaacctggattgttgagagcaaagaatgcatcaaagaagctgattgaattagggttagagttcactccagcagaagaaattatcaaggatgcagttgagtgtttgaagagtagaggtttggtttaa

SEQ ID NO: 4 - DNA, 1255 bp, Medicago truncatula
  source 1..1255: mol_type = genomic DNA
atgcattttttgtagagctaaaagaaaaaggaaaaaaaaaacaagaaagaaaaacatggcaggaaacaaaattccagaagtgttattgaattcaggacacaaaatgccagtcataggaatgggaacttcagtagacaatcgtccatcaaatgatgttcttgcttcaatctttgttgatgcaatcaaagttggttatcgccattttgattctgcttctgtgtatggaacagaagaagccataggtatggctgtggcaaaagctttagaacaaggtcttattaagagtagagatgaacttttcatcacttcaaagccatggaacactgatgcagattatgatcttattgttccagctctcaaaaccacattaaaaaaactgggaacggagtatgtagatctttatctgattcattggccagtaagactgagacatgatcttgaaaacccagtcatatttaccaaagaagatttacttccctttgatatagaagggacatggaaagctatggaagagtgttataagttaggcttagcaaagtccattggcatatgcaattatggtaccaaaaaattgactaaactcttggaaactgctaccatcacccctgcagtgaatcaggtggagatgaatccttcttggcagcaagggaaactgagggaattttgcaaggagaaaggaattcatgttagtgcttggtcagctcttggagcttataaggttacttggggttcaggagctgtcgtggagaatcaaattcttcaagacatagcagctgctaaagggaagactacagctcaggttgcactcagatgggtgtaccaaataggatcaagtgcaatggccaaaagctttaacaaggagaggatgacacaaaaccttgaaatatttgattttgagctgagtgaagatgatttggagaagattaagcagattccacaacgcaggcaatacttaggtgatatgtggctatcggaaaatggatcttgcaagaccttagaagaactttgggatggagatgtttgaaaatttcctcttaagtcctaactatattaaaggaaaataaagttcatgatttgaaaattattatgtatcagcttttcttatttcacaagtgtccttgtttgagaccttgagttgaccaagaatgttagtgtgacattcatatatgtagcctcagttatgtggctctgcataatttgttccaacttcaaataaagaaaagttttattctcaaaaaaaaaaaaaaaaaaaaaa

SEQ ID NO: 5 - DNA, 960 bp, synthetic construct
  source 1..960: mol_type = other DNA
atgtccaagaccgtgtgcgtgaccggtgcctccggtgcaatcggctcctgggttgtgcgcctgctgctggaacgcggttacaccgtgcacgcaaccatccaggatctggaagatgaaaacgaaaccaagcacctggaagcaatggaaggcgcaaagacccgcttgaagttcttcgaaatggatctgctgaactccgattccattgcagcagcagtgaagggctgcgcaggcgtgatccacctggcatgcccaaacatcatcggcgaagtgaaggacccagaaaagcagatcctcgaaccagcaatccagggcaccgtgaacgtgctgaaggtggcaaaagaagcaggcgtcgaacgcgtggtggcaacctcctccatctccgcaatcatcccatctccatcctggccagcagataagatcaaggcagaagattgctggaccgatctggaatactgcaaagaaaagaagctgtactacccaatcgctaagaccctggcagaaaaggcaggctgggagttcgcaaaagaaaccggcttcgatgtggtgatgatcaacccaggcaccgcactgggtccactgatcccaccacgcatcaactcctctatggcagtgctggcaggcgtcctgaagggcgataaagaaacctacgaagatttcttcatgggcatggcacacttcaaggatatcgcactggcacacatcctgggcttcgaacagaagaaggcatccggtcgccacctgtgcgtggaagccatccgccactactccgatttcgtgaacctggtggcagaactgtacccagaatacaacgtggcaaagatcccaaccgatactcagccaggcctgcttcgcgcaaagaacgcatccaagaagctgatcgaactgggcctcgaatttaccccagccgaagaaatcatcaaggatgcagtggaatgcctgaagtcccgtggcctggtgtaa

SEQ ID NO: 6 - DNA, 969 bp, synthetic construct
  source 1..969: mol_type = other DNA
atggcaggcaacaagatcccagaagtgctgctgaactccggtcacaagatgccagtgatcggcatgggcacctccgtggataaccgtccatccaacgatgtgctggcatccatcttcgtggatgcaatcaaggtgggctaccgccacttcgattccgcatccgtgtacggcaccgaagaggcaatcggtatggcagtggcaaaggcactggaacagggcctgatcaagtcccgtgatgaactcttcatcacctccaagccttggaacaccgatgcagattacgatctgatcgtgccagcactcaagaccaccttgaagaagctgggcaccgaatacgtggatctgtacctgatccactggcctgtgcgcctgcgccacgatctggaaaacccagtgatcttcaccaaagaagatctgctgccattcgacatcgaaggcacctggaaggcaatggaagaatgctacaagctgggcctcgcaaagtccatcggcatctgcaactacggcaccaaaaagctgaccaagctgctggaaaccgcaaccatcactccagcagtgaaccaggtggaaatgaacccatcctggcagcagggcaagctgcgcgagttctgcaaagaaaagggcatccacgtgtccgcatggtccgcactgggtgcatacaaggtgacctggggctccggtgcagtggtggaaaaccagatcctccaggatatcgcagcagcaaagggtaagaccaccgcacaggtggcactgcgctgggtgtaccagatcggctcctccgcaatggcaaagtccttcaacaaagaacgcatgacccagaacctggaaatcttcgatttcgaactgtccgaagatgatctcgaaaagatcaagcagatcccacagcgtcgccagtacctgggcgatatgtggctgtccgaaaacggctcctgcaagaccctggaagaactgtgggatggcgacgtgtaa

SEQ ID NO: 7 - protein, 491 aa, Corynebacterium glutamicum
MASTFIQADSPEKSKKLPPLTEGPYRKRLFYVALVATFGGLLFGYDTGVINGALNPMTRELGLTAFTEGVVTSSLLFGAAAGAMFFGRISDNWGRRKTIISLAVAFFVGTMICVFAPSFAVMVVGRVLLGLAVGGASTVVPVYLAELAPFEIRGSLAGRNELMIVVGQLAAFVINAIIGNVFGHHDGVWRYMLAIAAIPAIALFFGMLRVPESPRWLVERGRIDEARAVLETIRPLERAHAEVADVEHLAREEHAVSEKSMGLREILSSKWLVRILLVGIGLGVAQQLTGINSIMYYGQVVLIEAGFSENAALIANVAPGVIAVVGAFIALWMMDRINRRTTLITGYSLTTISHVLIGIASVAFPVGDPLRPYVILTLVVVFVGSMQTFLNVATWVMLSELFPLAMRGFAIGISVFFLWIANAFLGLFFPTIMEAVGLTGTFFMFAGIGVVALIFIYTQVPETRGRTLEEIDEDVTSGVIFNKDIRKGKVH

SEQ ID NO: 8 - protein, 508 aa, Corynebacterium glutamicum
MTDIKATSSTSATTAPTAGRPARRLGQISLVACLGGLLFGYDTGVANGAEGHMAQELGLNVLQLGVVISSLVFAAAFGALFAGRISDEIGRRKAIITLSVLFFLGSILVVFSPAGELGQFYGPGFATLVTGRIMLGLAVGGASTVVPVYLAELAPLEIRGSLTGRNELAIVTGQLLAFVINALIAVTLHGVIDGIWRIMFAVCALPAVALFLGMLRMPESPRWLVNQGRYDDARRVMETVRTPERAKAEMDEIIAVHSENNAALPGVKQSSGQASGQVSSKHTHMSIGEVLSNKWLVRLLIAGIGVAVAQQLTGINAIMYYGTRVLEESGMSAEMAVVANIAFGAVAVIGGLIALRNMDRLDRRTTFIIGLSLTTTFHLLIAAAGTLLPEGNSIRPFAIMILVVGFVLSMQTFLNVAVWVWLAEIFPVRMKGIGTGISVFCGWGINGVLALFFPALVSGVGITFSFLIFAVVGVIALAFVTKFVPETRGRSLEELDHAAFTGQIFKKA

SEQ ID NO: 9 - DNA, 1473 bp, Corynebacterium glutamicum
  source 1..1473: mol_type = genomic DNA
atggctagtaccttcattcaggccgacagccctgaaaaaagtaagaagctgcccccactcacagaaggtccgtatagaaagcggctattctacgttgcactagttgcgacgtttggtgggctgctcttcggatatgacaccggagtaatcaacggtgcactcaacccaatgacacgtgagctcggactaaccgcgttcaccgagggtgttgtaacttcttccctgctgtttggtgcagcagctggtgcgatgtttttcggtcgcatttccgacaactggggtcgccggaaaacaatcatctcacttgcagtagctttctttgtcggcaccatgatctgcgtgtttgctccatcttttgcagtaatggttgtcggacgtgtgcttcttggactcgcagttggtggcgcttccactgttgtccctgtctacctggctgaacttgctccttttgaaatccgtggctcactggctggccgtaatgagttgatgattgttgttggtcagctcgcagcttttgtcatcaatgcgattattggaaatgtttttggacaccacgatggtgtgtggcgctacatgctggcaattgccgcaatcccagcaattgccctcttctttggaatgctccgagttccagaatccccacgctggcttgttgagcgaggacgcattgatgaggctcgcgcagttcttgaaaccattcgccctctagaacgtgcccatgcagaagttgctgatgttgaacacctagcaagagaagagcacgccgtttccgagaagtccatgggcttaagggaaattttgtccagcaagtggcttgtgcgcatcctcctggtaggtatcggattgggtgtcgcacagcagctgaccggcatcaactccatcatgtactacggccaggttgttctcattgaggctggtttctccgagaatgcagctctgatcgccaacgtggcgccaggagtgatcgcagttgtcggtgcattcatcgcactgtggatgatggatcgtatcaaccgccgtaccaccctcattaccggttattctctcaccaccattagccacgtattgatcggtatcgcatccgtagcattcccagtcggcgatcctcttcgcccctacgttatcttgactctggttgtggtcttcgtgggatccatgcagaccttcctcaacgtagctacctgggttatgctctctgagctcttcccgctggcaatgcgcggtttcgcaatcggtatctcagtgttcttcctctggatcgcaaacgcgttcctcggattgttcttcccaaccatcatggaagcagtaggactaaccggaaccttcttcatgttcgccggaatcggtgtggttgccttgatcttcatctacacccaggttcctgaaactcgtggacgtaccttggaggagattgatgaggatgttacttccggtgtcattttcaacaaggacatccgaaaaggaaaggtgcac

SEQ ID NO: 10 - DNA, 1527 bp, Corynebacterium glutamicum
  source 1..1527: mol_type = genomic DNA
atgacggacatcaaggccacatcaagtacatcggccactacagcaccaacagcaggccgaccagcgcgtcgacttggacaaatttccctcgtcgcctgtctcggcggacttctcttcggctatgacaccggtgtcgccaacggcgccgaaggccacatggcacaagaactcggactcaacgtgctgcagctcggcgttgtcatcagttcactggttttcgctgcagcctttggcgcgctgttcgctgggcgtatctcggacgaaatcgggcgtcgaaaagcaattatcactttgtccgtgctgttcttcctcggatcaatcctcgtcgtattctcccccgccggtgagctggggcagttctacggaccaggatttgccaccttggtcaccgggcgcatcatgttgggtctcgcggttggcggcgcctccacagtagttccggtgtacctcgctgaactcgcaccactagaaatccgcggctccctgaccggccgaaacgagcttgctatcgtcaccggccagctgcttgccttcgtgatcaacgcgcttatcgccgtcaccctacacggagttattgatggaatctggcgcatcatgttcgccgtctgtgccctccctgccgtcgccctcttcctcggcatgctgcggatgccggaatcaccacgctggctggtcaaccaggggcgttacgacgacgcccgccgcgtcatggagaccgtccgtacccctgagcgtgcgaaagccgaaatggatgaaatcatcgcggtgcactctgaaaacaatgcggcacttcctggtgttaagcagtcttcgggccaggcttcaggccaggtttctagcaagcacacccacatgtccatcggcgaagtcctcagcaacaaatggctggttcgtctgctcatcgccggcatcggtgttgcagttgcccagcagctcaccggcatcaacgccatcatgtactacggaacccgcgtcctcgaggaatccggcatgagcgcagaaatggctgtggttgccaacattgctttcggtgccgttgccgtcatcggtggactgatcgcactgcgcaacatggaccgcctggatcgccgcaccaccttcatcatcggcctgtcactgaccaccaccttccaccttttgatcgcagctgccggcactctccttccagaaggtaactccattcgaccattcgccatcatgatccttgttgttgggttcgtgctctccatgcagactttcctcaacgttgcagtgtgggtgtggctggcggaaatcttcccagtccgaatgaagggtatcggcaccggtatttcggtattctgcggttggggcatcaatggcgtcctagcgttgttcttcccagcactggtctccggcgtgggtatcaccttctccttccttatcttcgcagtcgtcggagtcattgccctggcgttcgtcaccaagtttgttcctgaaacccgtggccgctcacttgaagaactcgatcacgcagcattcaccggccagatcttcaagaaggcttaa

SEQ ID NO: 11 - protein, 363 aa, Corynebacterium glutamicum
MSTSTIRVAIAGVGNCATSLIQGVEYYRNADPSETVPGLMHVKFGDYHVGDIEFVAAFDVDAEKVGIDLADATEASQNCTIKIADVPQTGINVLRGPTLDGLGDHYRATIDESTAEPVDVVQALIDAKADVLVSYLPVGSEEADKFYAQAAIDAGCAFVNALPVFIASDPEWAKKFTDAGIPIVGDDIKSQIGATITHRVLARLFEERGVRVDRTMQLNVGGNMDFKNMLDRNRLESKKVSKTQAVTSNIPDGPLSGKVEDRNVHIGPSDHVQWLDDRKWAYVRLEGTAFGGVPLNLEYKLEVWDSPNSAGIIIDAVRAAKIALDRGIGGPIMPASSYLMKSPPEQLPDDVARERLEAFIIEA

SEQ ID NO: 12 - DNA, 1092 bp, Corynebacterium glutamicum
  source 1..1092: mol_type = genomic DNA
atgagcacgtccaccatcagggttgccattgccggagtcggaaactgcgcgacctccctcattcagggtgtggaatattaccgaaatgcggatccttccgaaactgtcccgggtttgatgcacgtcaaattcggtgattaccacgttggcgacattgaattcgtggccgcgttcgacgtcgacgccgaaaaagtaggcatcgatcttgccgacgccaccgaggcttcacaaaactgcactatcaaaatcgccgatgtcccacagaccggcatcaacgtgctgcgtggcccgactctcgacggcctgggcgatcattaccgcgcgaccatcgacgagtccaccgccgagccagtcgacgttgtccaggcgcttatcgacgcaaaagccgatgttttggtgtcctacctcccagtgggctccgaagaagccgacaaattctacgcacaagccgccatcgatgcaggctgcgcctttgtcaacgctctcccagtattcatcgcctccgaccctgagtgggctaagaagttcactgacgctggcatcccaattgttggcgatgacatcaaatcccagatcggtgcaaccatcacccaccgtgtcctcgcacgcctttttgaagaacgtggcgttcgcgtagatcgcaccatgcagctcaacgtcggcggcaacatggacttcaaaaacatgcttgaccgcaatcgcttggaatccaagaaggtctccaaaacccaagcagtgacctccaacattccagatggtccactgtctggaaaggtggaagaccgcaacgtccacatcggaccatccgaccacgtccaatggctcgatgaccgcaagtgggcttatgtccgcctcgaaggcaccgcattcggtggagttcccctcaaccttgagtacaaactcgaggtgtgggattcacccaactctgccggcatcatcatcgacgctgttcgcgccgccaagatcgccctcgatcgcggtatcggcggaccgatcatgccagcaagctcctacctgatgaagtccccacctgagcagcttccagacgatgttgctcgtgaacgcctagaggcattcatcatcgaggcgtaa

SEQ ID NO: 13 - protein, 275 aa, Corynebacterium glutamicum
MDARGMLAIAEAVVDDAEALFMQGFGAAPAHMKSPGDFATEVDMAIESHMRSMLNMMTGIAVIGEEGGGATSGTRWVIDPIDGTANFAASNPMSAILVSLLVDDQPVLGITSMPMLGKRLTAFEGSPLMINGEPQEPLQEQSSLVSHIGFSSMASPRNTAFPVELRRDLLTELTESYLRPRITGSVGVDLAFTAQGIFGACVSFSPHVWDNSAGVMLMRAAGAQVTDTEGHPWAPGRGVVAGTKRAHDVLLSKIEKVRLMHADAGNDQSLNEEYK

SEQ ID NO: 14 - DNA, 828 bp, Corynebacterium glutamicum
  source 1..828: mol_type = genomic DNA
atggatgctcgtgggatgttggccattgcggaggccgttgtagatgatgccgaagccctcttcatgcagggcttcggagctgcacctgcccatatgaaatccccgggggattttgccacggaagtggatatggccatcgaatcccatatgcgttcgatgctgaacatgatgacaggcattgctgtcatcggtgaagaaggtggcggtgcgacctccggcacgcgctgggtgattgatcccatcgacggcaccgccaacttcgcggcgtccaacccgatgagcgcgatcctggtgtctttgcttgtcgacgaccagcccgtcctgggtattacctccatgcccatgctgggtaaacgcctcaccgcttttgaaggttcaccgctgatgatcaacggtgaacctcaggaaccattgcaagaacaatccagtttggtatcccacattggttttagttccatggcctccccgcgcaatacagcgtttcctgtggagttgcgtcgggatcttctgaccgagctcacggaatcgtatcttcgtccccgcattacaggttcggtgggtgttgatctcgcgttcactgcgcagggcatttttggagcatgcgtatcgtttagtcctcatgtttgggacaattccgcaggcgtgatgttgatgcgcgctgctggtgcacaagttactgacaccgaaggccatccgtgggcaccaggtaggggagtcgtggccggaacaaaaagggctcacgatgtgctgttaagtaagattgaaaaagttcggttgatgcatgcagatgcaggtaatgaccagtcgttaaatgaggagtacaagtaa

SEQ ID NO: 15 - DNA, 2013 bp, synthetic construct
  source 1..2013: mol_type = other DNA
ctcaagcggaacctgaaggatgaagggctaaaaggtgtcttcacgattgtgaggaacgtgattagccaaccggatctgcgcaagcgagtgctcggaatgcgaaagactttcaccgagcataaagatcacttaggtgcggttggcatcattttgcagaagagagcccaatagggatctgaaatggaggggtgcgtcgataagcaatttagaccgtgaacgctgacttcaacgcctgcagcgcgtcgctggagtcgcccgatgcccacgcctccatgccgatgacgccgtcgtagcccatcgcggcgagagctttcgcgacgccctggtagttgatctcgccggtgccgggttccatgcggccggggacatcggcaacctggatttcgccgatgaatggctgcgcctcacggagcagctcaatgaggtttccttcgccaatctgggcgtggtacaaatccaggttgaggcgcagattcgggtgattgacagccttgaccagcgccaaagtgtcagtggccttggcaaaaggagtgccggggtgatcgactgcgaggttgaggttttccagcacgaaaaccttgcctgcgcgctcccccagctcagcgatctggcggagcgtttcagcagcgtagagccacatttctggggtaaccacttcaatgggagtaacaggtagtccctgcggtccaaggccagttccatgcagattcagccgggggcagttgagcttttccgccaccgccaaggactccgaagcggttgccaagagctccgcgcggccctgttcagtaatcagatccccgcgcaggtagcccgtcatggaggaaaattccgcgcctgttgccacgagcgcatcgatgtcttttgtggaccagtcccaaatttccacgaggaatccctgatcagagatcgtcttgaccctctcctcgaaaggcaggtcctggtagatcatctctgcgcatgctgcgagtttaaaagtcatggttaaacctcgatgctttcagcaaggagggcaagtttgactgacatttttcatccttccaagttttactagaacgttctactataacgttctagtagatactagataccacccattgatgccgtcaaggggtttcctgtaaagatgtaagagattaagaaaaagaggtagatatggcgtcaaagcgaccgacaatggctgatgtggcaaaagctgctggagtatccactgcgctggtctccatcgtgtttcgcgatgcccccggagcaagtgaatccacccgcaaccatgtgaaagaaaaagccgccgaactcggatacattcctgatcgacgagcccaaaaacttcgccaaaaccgctccggactcatcggtgtggcattcgaaatgcaccaagcattccacggcgatatcgtcgaacacctctatcccaccgcccgaaaacatggcttcgacctgtaccttagcgcgatcacaccgactcgcactgaaaaagatgccgtcaacgccctgatcagggaacgatgcgaagcagtaattcttctaggatctcgcatgtcacctagtgatttggaaacaatcgcacagcaacttcccgtccaagtaattgcccgcggttccggaacccccaaagtcagttccgtccatgtcgacgacgcagttggcgcccaattagccctcaaccacctcatcgaattaggccacgaacacatcatctacatcgatggtggcgacgcccctggcacccaggaacgatcagaagtgttcaaagcgcacattgattccttcgccggcaccacccgcatagtccctggtggcagcagcgaagcagcaggagcccaagcaatctcagagattctggattccggaactgacgccaccgccatcctcgcattcaatgaccgagtagccctcggcgtgctcgacatcttatggcagcgcggcatccacgtccccgaagaaatctccgtggtgggatacgacaactcaagccttgccagcctcgaccacatcggcttgaccaccataatt

SEQ ID NO: 16 - DNA, 40 bp, synthetic construct
  source 1..40: mol_type = other DNA
gaggatccccgggtaccgagctcgttccgccaactcaacc

SEQ ID NO: 17 - DNA, 26 bp, synthetic construct
  source 1..26: mol_type = other DNA
tgaaaccactctggtggccaggtaag

SEQ ID NO: 18 - DNA, 43 bp, synthetic construct
  source 1..43: mol_type = other DNA
cttacctggccaccagagtggtttcagaagagtccctggtttc

SEQ ID NO: 19 - DNA, 43 bp, synthetic construct
  source 1..43: mol_type = other DNA
cgttgtaaaacgacggccagtgaatttccttggtcaccagatc

SEQ ID NO: 20 - DNA, 43 bp, synthetic construct
  source 1..43: mol_type = other DNA
gaggatccccgggtaccgagctcgggaacccaattcaccttcg

SEQ ID NO: 21 - DNA, 18 bp, synthetic construct
  source 1..18: mol_type = other DNA
gcctagcaggccaacaac

SEQ ID NO: 22 - DNA, 41 bp, synthetic construct
  source 1..41: mol_type = other DNA
aaattgttgttggcctgctaggctgcgctggttccatctgc

SEQ ID NO: 23 - DNA, 44 bp, synthetic construct
  source 1..44: mol_type = other DNA
cgttgtaaaacgacggccagtgaattggaccaaccagaaacttc

SEQ ID NO: 24 - DNA, 24 bp, synthetic construct
  source 1..24: mol_type = other DNA
agcggataacaatttcacacagga

SEQ ID NO: 25 - DNA, 21 bp, synthetic construct
  source 1..21: mol_type = other DNA
cgccagggttttcccagtcac

SEQ ID NO: 26 - DNA, 17 bp, synthetic construct
  source 1..17: mol_type = other DNA
gggatttcgttgccatg

SEQ ID NO: 27 - DNA, 17 bp, synthetic construct
  source 1..17: mol_type = other DNA
ggttgcggcaatcttcc

SEQ ID NO: 28 - DNA, 16 bp, synthetic construct
  source 1..16: mol_type = other DNA
acaccatccgggacac

SEQ ID NO: 29 - DNA, 16 bp, synthetic construct
  source 1..16: mol_type = other DNA
cgttcaagacgtcatc

SEQ ID NO: 30 - DNA, 42 bp, synthetic construct
  source 1..42: mol_type = other DNA
gaggatccccgggtaccgagctcggaatctgactccgagcag

SEQ ID NO: 31 - DNA, 18 bp, synthetic construct
  source 1..18: mol_type = other DNA
aagtcagcgttcacggtc

SEQ ID NO: 32 - DNA, 42 bp, synthetic construct
  source 1..42: mol_type = other DNA
atttagaccgtgaacgctgacttgagggcaagtttgactgac

SEQ ID NO: 33 - DNA, 44 bp, synthetic construct
  source 1..44: mol_type = other DNA
cgttgtaaaacgacggccagtgaattatggtggtcaagccgatg

SEQ ID NO: 34 - DNA, 19 bp, synthetic construct
  source 1..19: mol_type = other DNA
gttccatcaaagtcaatgc

SEQ ID NO: 35 - DNA, 19 bp, synthetic construct
  source 1..19: mol_type = other DNA
gtgcgccgtgtgatcaatg

SEQ ID NO: 36 - DNA, 43 bp, synthetic construct
  source 1..43: mol_type = other DNA
tttaactttaagaaggagatataccatgtccaagaccgtgtgc

SEQ ID NO: 37 - DNA, 39 bp, synthetic construct
  source 1..39: mol_type = other DNA
gcaggtgcacaatgatacgattacaccaggccacgggac

SEQ ID NO: 38 - DNA, 45 bp, synthetic construct
  source 1..45: mol_type = other DNA
tttaactttaagaaggagatataccatggcaggcaacaagatccc

SEQ ID NO: 39 - DNA, 44 bp, synthetic construct
  source 1..44: mol_type = other DNA
tggcaccagagcgagctctgcggccttacacgtcgccatcccac

SEQ ID NO: 40 - DNA, 40 bp, synthetic construct
  source 1..40: mol_type = other DNA
ctttaagaaggagatataccatgagcacgtccaccatcag

SEQ ID NO: 41 - DNA, 40 bp, synthetic construct
  source 1..40: mol_type = other DNA
acatcgttgagtggtcaccgttacgcctcgatgatgaatg

SEQ ID NO: 42 - DNA, 49 bp, synthetic construct
  source 1..49: mol_type = other DNA
cggtgaccactcaacgatgtgaaggagatataccatgtccaagaccgtg

SEQ ID NO: 43 - DNA, 44 bp, synthetic construct; identical to SEQ ID NO: 39
  source 1..44: mol_type = other DNA

SEQ ID NO: 44 - DNA, 46 bp, synthetic construct
  source 1..46: mol_type = other DNA
tcgggctcatgagcgcttgtttcggtaatcgtattgtacacggccg

SEQ ID NO: 45 - DNA, 43 bp, synthetic construct
  source 1..43: mol_type = other DNA
cggccacggggcctgccaccatacatccggatatagttcctcc

SEQ ID NO: 46 - DNA, 18 bp, synthetic construct
  source 1..18: mol_type = other DNA
ccgaaacaagcgctcatg

SEQ ID NO: 47 - DNA, 20 bp, synthetic construct
  source 1..20: mol_type = other DNA
gtatggtggcaggccccgtg

SEQ ID NO: 48 - DNA, 40 bp, synthetic construct; identical to SEQ ID NO: 40
  source 1..40: mol_type = other DNA

SEQ ID NO: 49 - DNA, 43 bp, synthetic construct
  source 1..43: mol_type = other DNA
gcaccagagcgagctctgcggccttacgcctcgatgatgaatg

SEQ ID NO: 50 - DNA, 43 bp, synthetic construct
  source 1..43: mol_type = other DNA
gttaagtataagaaggagatatacaatgtccaagaccgtgtgc

SEQ ID NO: 51 - DNA, 44 bp, synthetic construct
  source 1..44: mol_type = other DNA
cgatatccaattgagatctgccatattacacgtcgccatcccac